European Patent Specification EP 4 211 231 B1, published June 26, 2024. Title: PEPTIDE-MODIFIED AAV CAPSID. Applicant: GENETHON INSTITUT NATIONAL DE LA RECHERCHE ET DE LA SANTE MEDICALE UNIVERSITE D'EVRY VAL D'ESSONNE. The sequence listing filed with the application follows.

SEQUENCE LISTING (42 sequences)

SEQ ID NO: 1 - protein, 7 aa, artificial sequence
  synthetic peptide (P1)
RGDLGLS

SEQ ID NO: 2 - protein, 737 aa, artificial sequence
  synthetic polypeptide (AAV9.rh74)
MAADGYLPDWLEDNLSEGIREWWALKPGAPQPKANQQHQDNARGLVLPGYKYLGPGNGLDKGEPVNAADAAALEHDKAYDQQLKAGDNPYLKYNHADAEFQERLKEDTSFGGNLGRAVFQAKKRLLEPLGLVEEAAKTAPGKKRPVEQSPQEPDSSAGIGKSGAQPAKKRLNFGQTGDTESVPDPQPIGEPPAAPSGVGSLTMASGGGAPVADNNEGADGVGSSSGNWHCDSQWLGDRVITTSTRTWALPTYNNHLYKQISNSTSGGSSNDNAYFGYSTPWGYFDFNRFHCHFSPRDWQRLINNNWGFRPKRLNFKLFNIQVKEVTDNNGVKTIANNLTSTVQVFTDSDYQLPYVLGSAHEGCLPPFPADVFMIPQYGYLTLNDGSQAVGRSSFYCLEYFPSQMLRTGNNFQFSYEFENVPFHSSYAHSQSLDRLMNPLIDQYLYYLSRTQSTGGTAGTQQLLFSQAGPNNMSAQAKNWLPGPCYRQQRVSTTLSQNNNSNFAWTGATKYHLNGRDSLVNPGVAMATHKDDEERFFPSSGVLMFGKQGAGKDNVDYSSVMLTSEEEIKTTNPVATEQYGVVADNLQQQNAAPIVGAVNSQGALPGMVWQNRDVYLQGPIWAKIPHTDGNFHPSPLMGGFGMKHPPPQILIKNTPVPADPPTAFNKDKLNSFITQYSTGQVSVEIEWELQKENSKRWNPEIQYTSNYYKSNNVEFAVNTEGVYSEPRPIGTRYLTRNL

SEQ ID NO: 3 - DNA, 2214 bp, artificial sequence
  synthetic polynucleotide (AAV9.rh74)
  CDS (1)..(2214)
atggctgccgatggttatcttccagattggctcgaggacaaccttagtgaaggaattcgcgagtggtgggctttgaaacctggagcccctcaacccaaggcaaatcaacaacatcaagacaacgctcgaggtcttgtgcttccgggttacaaataccttggacccggcaacggactcgacaagggggagccggtcaacgcagcagacgcggcggccctcgagcacgacaaggcctacgaccagcagctcaaggccggagacaacccgtacctcaagtacaaccacgccgacgccgagttccaggagcggctcaaagaagatacgtcttttgggggcaacctcgggcgagcagtcttccaggccaaaaagaggcttcttgaacctcttggtctggttgaggaagcggctaagacggctcctggaaagaagaggcctgtagagcagtctcctcaggaaccggactcctccgcgggtattggcaaatcgggtgcacagcccgctaaaaagagactcaatttcggtcagactggcgacacagagtcagtcccagaccctcaaccaatcggagaacctcccgcagccccctcaggtgtgggatctcttacaatggcttcaggtggtggcgcaccagtggcagacaataacgaaggtgccgatggagtgggtagttcctcgggaaattggcattgcgattcccaatggctgggggacagagtcatcaccaccagcacccgaacctgggccctgcccacctacaacaatcacctctacaagcaaatctccaacagcacatctggaggatcttcaaatgacaacgcctacttcggctacagcaccccctgggggtattttgacttcaacagattccactgccacttctcaccacgtgactggcagcgactcatcaacaacaactggggattccggcctaagcgactcaacttcaagctcttcaacattcaggtcaaagaggttacggacaacaatggagtcaagaccatcgccaataaccttaccagcacggtccaggtcttcacggactcagactatcagctcccgtacgtgctcgggtcggctcacgagggctgcctcccgccgttcccagcggacgttttcatgattcctcagtacgggtatctgacgcttaatgatggaagccaggccgtgggtcgttcgtccttttactgcctggaatatttcccgtcgcaaatgctaagaacgggtaacaacttccagttcagctacgagtttgagaacgtacctttccatagcagctacgctcacagccaaagcctggaccgactaatgaatccactcatcgaccaatacttgtactatctctcacggactcaaagcacgggcggtactgcaggaactcagcagttgctattttctcaggccgggcctaacaacatgtcggctcaggccaagaactggctacccggtccctgctaccggcagcaacgcgtctccacgacactgtcgcagaacaacaacagcaactttgcctggacgggtgccaccaagtatcatctgaatggcagagactctctggtgaatcctggcgttgccatggctacccacaaggacgacgaagagcgattttttccatccagcggagtcttaatgtttgggaaacagggagctggaaaagacaacgtggactatagcagcgtgatgctaaccagcgaggaagaaataaagaccaccaacccagtggccacagaacagtacggcgtggtggccgataacctgcaacagcaaaacgccgctcctattgtaggggccgtcaatagtcaaggagccttacctggcatggtgtggcagaacagagatgtgtacctgcaaggacccatttgggccaaaattcctcacacggacggcaactttcacccttctccgctgatgggagggtttggaatgaagcacccgcctcctcagatcctcatcaaaaacacacctgtacctgcggatcctccaacggccttcaacaaggacaagctgaactctttcatcacccagtattctactggccaagtcagcgtggagatcgagtgggagctgcagaaggaaaacagcaagcgctggaacccggagatccagtacacttccaactattacaagtctaataatgttgaatttgctgttaatactgaaggtgtatatagtgaaccccgccccattggcaccagatacctgactcgtaatctgtaa

SEQ ID NO: 4 - protein, 737 aa, artificial sequence; identical to SEQ ID NO: 2
  Synthetic Construct

SEQ ID NO: 5 - protein, 12 aa, artificial sequence
  synthetic peptide
AAARGDLGLSSG

SEQ ID NO: 6 - protein, 749 aa, artificial sequence
  synthetic polypeptide (AAV9-rh74-HB-P1)
MAADGYLPDWLEDNLSEGIREWWALKPGAPQPKANQQHQDNARGLVLPGYKYLGPGNGLDKGEPVNAADAAALEHDKAYDQQLKAGDNPYLKYNHADAEFQERLKEDTSFGGNLGRAVFQAKKRLLEPLGLVEEAAKTAPGKKRPVEQSPQEPDSSAGIGKSGAQPAKKRLNFGQTGDTESVPDPQPIGEPPAAPSGVGSLTMASGGGAPVADNNEGADGVGSSSGNWHCDSQWLGDRVITTSTRTWALPTYNNHLYKQISNSTSGGSSNDNAYFGYSTPWGYFDFNRFHCHFSPRDWQRLINNNWGFRPKRLNFKLFNIQVKEVTDNNGVKTIANNLTSTVQVFTDSDYQLPYVLGSAHEGCLPPFPADVFMIPQYGYLTLNDGSQAVGRSSFYCLEYFPSQMLRTGNNFQFSYEFENVPFHSSYAHSQSLDRLMNPLIDQYLYYLSRTQSTGGTAGTQQLLFSQAGPNNMSAQAKNWLPGPCYRQQRVSTTLSQNNNSNFAWTGATKYHLNGRDSLVNPGVAMATHKDDEERFFPSSGVLMFGKQGAGKDNVDYSSVMLTSEEEIKTTNPVATEQYGVVADNLQQQNAAARGDLGLSSGAAPIVGAVNSQGALPGMVWQNRDVYLQGPIWAKIPHTDGNFHPSPLMGGFGMKHPPPQILIKNTPVPADPPTAFNKDKLNSFITQYSTGQVSVEIEWELQKENSKRWNPEIQYTSNYYKSNNVEFAVNTEGVYSEPRPIGTRYLTRNL

SEQ ID NO: 7 - DNA, 2250 bp, artificial sequence
  synthetic polynucleotide (AAV9-rh74-HB-P1)
  CDS (1)..(2250)
atggctgccgatggttatcttccagattggctcgaggacaaccttagtgaaggaattcgcgagtggtgggctttgaaacctggagcccctcaacccaaggcaaatcaacaacatcaagacaacgctcgaggtcttgtgcttccgggttacaaataccttggacccggcaacggactcgacaagggggagccggtcaacgcagcagacgcggcggccctcgagcacgacaaggcctacgaccagcagctcaaggccggagacaacccgtacctcaagtacaaccacgccgacgccgagttccaggagcggctcaaagaagatacgtcttttgggggcaacctcgggcgagcagtcttccaggccaaaaagaggcttcttgaacctcttggtctggttgaggaagcggctaagacggctcctggaaagaagaggcctgtagagcagtctcctcaggaaccggactcctccgcgggtattggcaaatcgggtgcacagcccgctaaaaagagactcaatttcggtcagactggcgacacagagtcagtcccagaccctcaaccaatcggagaacctcccgcagccccctcaggtgtgggatctcttacaatggcttcaggtggtggcgcaccagtggcagacaataacgaaggtgccgatggagtgggtagttcctcgggaaattggcattgcgattcccaatggctgggggacagagtcatcaccaccagcacccgaacctgggccctgcccacctacaacaatcacctctacaagcaaatctccaacagcacatctggaggatcttcaaatgacaacgcctacttcggctacagcaccccctgggggtattttgacttcaacagattccactgccacttctcaccacgtgactggcagcgactcatcaacaacaactggggattccggcctaagcgactcaacttcaagctcttcaacattcaggtcaaagaggttacggacaacaatggagtcaagaccatcgccaataaccttaccagcacggtccaggtcttcacggactcagactatcagctcccgtacgtgctcgggtcggctcacgagggctgcctcccgccgttcccagcggacgttttcatgattcctcagtacgggtatctgacgcttaatgatggaagccaggccgtgggtcgttcgtccttttactgcctggaatatttcccgtcgcaaatgctaagaacgggtaacaacttccagttcagctacgagtttgagaacgtacctttccatagcagctacgctcacagccaaagcctggaccgactaatgaatccactcatcgaccaatacttgtactatctctcacggactcaaagcacgggcggtactgcaggaactcagcagttgctattttctcaggccgggcctaacaacatgtcggctcaggccaagaactggctacccggtccctgctaccggcagcaacgcgtctccacgacactgtcgcagaacaacaacagcaactttgcctggacgggtgccaccaagtatcatctgaatggcagagactctctggtgaatcctggcgttgccatggctacccacaaggacgacgaagagcgattttttccatccagcggagtcttaatgtttgggaaacagggagctggaaaagacaacgtggactatagcagcgtgatgctaaccagcgaggaagaaataaagaccaccaacccagtggccacagaacagtacggcgtggtggccgataacctgcaacagcaaaacgcggccgcccgcggcgatctgggcctgagctccggagccgctcctattgtaggggccgtcaatagtcaaggagccttacctggcatggtgtggcagaacagagatgtgtacctgcaaggacccatttgggccaaaattcctcacacggacggcaactttcacccttctccgctgatgggagggtttggaatgaagcacccgcctcctcagatcctcatcaaaaacacacctgtacctgcggatcctccaacggccttcaacaaggacaagctgaactctttcatcacccagtattctactggccaagtcagcgtggagatcgagtgggagctgcagaaggaaaacagcaagcgctggaacccggagatccagtacacttccaactattacaagtctaataatgttgaatttgctgttaatactgaaggtgtatatagtgaaccccgccccattggcaccagatacctgactcgtaatctgtaa

SEQ ID NO: 8 - protein, 749 aa, artificial sequence; identical to SEQ ID NO: 6
  Synthetic Construct

SEQ ID NO: 9 - protein, 15 aa, artificial sequence
  synthetic peptide (K-P1)
GQSGRGDLGLSAQAA

SEQ ID NO: 10 - DNA, 355 bp, artificial sequence
  synthetic polynucleotide (MscI fragment HB-P1)
tggccacagaacagtacggcgtggtggccgataacctgcaacagcaaaacgcggccgcccgcggcgatctgggcctgagctccggagccgctcctattgtaggggccgtcaatagtcaaggagccttacctggcatggtgtggcagaacagagatgtgtacctgcaaggacccatttgggccaaaattcctcacacggacggcaactttcacccttctccgctgatgggagggtttggaatgaagcacccgcctcctcagatcctcatcaaaaacacacctgtacctgcggatcctccaacggccttcaacaaggacaagctgaactctttcatcacccagtattctactggcca

SEQ ID NO: 11 - DNA, 346 bp, artificial sequence
  synthetic polynucleotide (MscI fragment K-P1)
tggccacagaacagtacggcgtggtggccgataacctgcaaggccagagcggccgcggcgatctgggcctgagcgcgcaggcggcgattgtaggggccgtcaatagtcaaggagccttacctggcatggtgtggcagaacagagatgtgtacctgcaaggacccatttgggccaaaattcctcacacggacggcaactttcacccttctccgctgatgggagggtttggaatgaagcacccgcctcctcagatcctcatcaaaaacacacctgtacctgcggatcctccaacggccttcaacaaggacaagctgaactctttcatcacccagtattctactggcca

SEQ ID NO: 12 - DNA, 2241 bp, artificial sequence
  synthetic polynucleotide (AAV9-rh74-K-P1)
  CDS (1)..(2241)
atggctgccgatggttatcttccagattggctcgaggacaaccttagtgaaggaattcgcgagtggtgggctttgaaacctggagcccctcaacccaaggcaaatcaacaacatcaagacaacgctcgaggtcttgtgcttccgggttacaaataccttggacccggcaacggactcgacaagggggagccggtcaacgcagcagacgcggcggccctcgagcacgacaaggcctacgaccagcagctcaaggccggagacaacccgtacctcaagtacaaccacgccgacgccgagttccaggagcggctcaaagaagatacgtcttttgggggcaacctcgggcgagcagtcttccaggccaaaaagaggcttcttgaacctcttggtctggttgaggaagcggctaagacggctcctggaaagaagaggcctgtagagcagtctcctcaggaaccggactcctccgcgggtattggcaaatcgggtgcacagcccgctaaaaagagactcaatttcggtcagactggcgacacagagtcagtcccagaccctcaaccaatcggagaacctcccgcagccccctcaggtgtgggatctcttacaatggcttcaggtggtggcgcaccagtggcagacaataacgaaggtgccgatggagtgggtagttcctcgggaaattggcattgcgattcccaatggctgggggacagagtcatcaccaccagcacccgaacctgggccctgcccacctacaacaatcacctctacaagcaaatctccaacagcacatctggaggatcttcaaatgacaacgcctacttcggctacagcaccccctgggggtattttgacttcaacagattccactgccacttctcaccacgtgactggcagcgactcatcaacaacaactggggattccggcctaagcgactcaacttcaagctcttcaacattcaggtcaaagaggttacggacaacaatggagtcaagaccatcgccaataaccttaccagcacggtccaggtcttcacggactcagactatcagctcccgtacgtgctcgggtcggctcacgagggctgcctcccgccgttcccagcggacgttttcatgattcctcagtacgggtatctgacgcttaatgatggaagccaggccgtgggtcgttcgtccttttactgcctggaatatttcccgtcgcaaatgctaagaacgggtaacaacttccagttcagctacgagtttgagaacgtacctttccatagcagctacgctcacagccaaagcctggaccgactaatgaatccactcatcgaccaatacttgtactatctctcacggactcaaagcacgggcggtactgcaggaactcagcagttgctattttctcaggccgggcctaacaacatgtcggctcaggccaagaactggctacccggtccctgctaccggcagcaacgcgtctccacgacactgtcgcagaacaacaacagcaactttgcctggacgggtgccaccaagtatcatctgaatggcagagactctctggtgaatcctggcgttgccatggctacccacaaggacgacgaagagcgattttttccatccagcggagtcttaatgtttgggaaacagggagctggaaaagacaacgtggactatagcagcgtgatgctaaccagcgaggaagaaataaagaccaccaacccagtggccacagaacagtacggcgtggtggccgataacctgcaaggccagagcggccgcggcgatctgggcctgagcgcgcaggcggcgattgtaggggccgtcaatagtcaaggagccttacctggcatggtgtggcagaacagagatgtgtacctgcaaggacccatttgggccaaaattcctcacacggacggcaactttcacccttctccgctgatgggagggtttggaatgaagcacccgcctcctcagatcctcatcaaaaacacacctgtacctgcggatcctccaacggccttcaacaaggacaagctgaactctttcatcacccagtattctactggccaagtcagcgtggagatcgagtgggagctgcagaaggaaaacagcaagcgctggaacccggagatccagtacacttccaactattacaagtctaataatgttgaatttgctgttaatactgaaggtgtatatagtgaaccccgccccattggcaccagatacctgactcgtaatctgtaa

SEQ ID NO: 13 - protein, 746 aa, artificial sequence
  Synthetic Construct
MAADGYLPDWLEDNLSEGIREWWALKPGAPQPKANQQHQDNARGLVLPGYKYLGPGNGLDKGEPVNAADAAALEHDKAYDQQLKAGDNPYLKYNHADAEFQERLKEDTSFGGNLGRAVFQAKKRLLEPLGLVEEAAKTAPGKKRPVEQSPQEPDSSAGIGKSGAQPAKKRLNFGQTGDTESVPDPQPIGEPPAAPSGVGSLTMASGGGAPVADNNEGADGVGSSSGNWHCDSQWLGDRVITTSTRTWALPTYNNHLYKQISNSTSGGSSNDNAYFGYSTPWGYFDFNRFHCHFSPRDWQRLINNNWGFRPKRLNFKLFNIQVKEVTDNNGVKTIANNLTSTVQVFTDSDYQLPYVLGSAHEGCLPPFPADVFMIPQYGYLTLNDGSQAVGRSSFYCLEYFPSQMLRTGNNFQFSYEFENVPFHSSYAHSQSLDRLMNPLIDQYLYYLSRTQSTGGTAGTQQLLFSQAGPNNMSAQAKNWLPGPCYRQQRVSTTLSQNNNSNFAWTGATKYHLNGRDSLVNPGVAMATHKDDEERFFPSSGVLMFGKQGAGKDNVDYSSVMLTSEEEIKTTNPVATEQYGVVADNLQGQSGRGDLGLSAQAAIVGAVNSQGALPGMVWQNRDVYLQGPIWAKIPHTDGNFHPSPLMGGFGMKHPPPQILIKNTPVPADPPTAFNKDKLNSFITQYSTGQVSVEIEWELQKENSKRWNPEIQYTSNYYKSNNVEFAVNTEGVYSEPRPIGTRYLTRNL

SEQ ID NO: 14 - protein, 746 aa, artificial sequence; identical to SEQ ID NO: 13
  synthetic polypeptide (AAV9-rh74-K-P1)

SEQ ID NO: 15 - DNA, 20 bp, artificial sequence
  synthetic oligonucleotide (Forward primer (CMV promoter))
catcaatgggcgtggatagc

SEQ ID NO: 16 - DNA, 24 bp, artificial sequence
  synthetic oligonucleotide (Reverse: Primer (CMV promoter))
ggagttgttacgacattttggaaa

SEQ ID NO: 17 - DNA, 18 bp, artificial sequence
  synthetic oligonucleotide (Probe (CMV promoter))
atttccaagtctccaccc

SEQ ID NO: 18 - DNA, 20 bp, artificial sequence
  synthetic oligonucleotide (Forward primer (Rplp0))
ctccaagcagatgcagcaga

SEQ ID NO: 19 - DNA, 20 bp, artificial sequence
  synthetic oligonucleotide (Reverse Primer (Rplp0))
atagccttgcgcatcatggt

SEQ ID NO: 20 - DNA, 22 bp, artificial sequence
  synthetic ooligonucleotide (Probe Rplp0) )
ccgtggtgctgatgggcaagaa

SEQ ID NO: 21 - protein, 12 aa, artificial sequence
  synthetic peptide
AAARGDLGLSAA

SEQ ID NO: 22 - DNA, 36 bp, artificial sequence
  synthetic polynucleotide
gcggccgccaggggcgacctgggcctgagcgcggcg

SEQ ID NO: 23 - protein, 12 aa, artificial sequence
  synthetic peptide
GSTRGDLGLSTG

SEQ ID NO: 24 - DNA, 36 bp, artificial sequence
  synthetic polynucleotide
ggcagcaccaggggcgacctgggcctgagcaccggc

SEQ ID NO: 25 - protein, 9 aa, artificial sequence
  synthetic peptide
GRGDLGLSG

SEQ ID NO: 26 - DNA, 27 bp, artificial sequence
  synthetic polynucleotide
ggcaggggcgacctgggcctgagcggc

SEQ ID NO: 27 - protein, 12 aa, artificial sequence
  synthetic peptide
SGSRGDLGLSGG

SEQ ID NO: 28 - DNA, 36 bp, artificial sequence
  synthetic polynucleotide
agcggcagcaggggcgacctgggcctgagcggcggc

SEQ ID NO: 29 - protein, 12 aa, artificial sequence
  synthetic peptide
SGARGDLGLSSA

SEQ ID NO: 30 - DNA, 36 bp, artificial sequence
  synthetic polynucleotide
agcggcgccaggggcgacctgggcctgagcagcgcg

SEQ ID NO: 31 - protein, 12 aa, artificial sequence
  synthetic peptide
SGARGDLGLSAG

SEQ ID NO: 32 - DNA, 36 bp, artificial sequence
  synthetic polynucleotide
agcggcgccaggggcgacctgggcctgagcgccggc

SEQ ID NO: 33 - protein, 12 aa, artificial sequence
  synthetic peptide
AGARGDLGLSSG

SEQ ID NO: 34 - DNA, 36 bp, artificial sequence
  synthetic polynucleotide
gcgggcgcgaggggcgacctgggcctgagcagcggc

SEQ ID NO: 35 - protein, 12 aa, artificial sequence
  synthetic peptide
GAARGDLGLSGA

SEQ ID NO: 36 - DNA, 36 bp, artificial sequence
  synthetic polynucleotide
ggcgcggcgaggggcgacctgggcctgagcggcgcg

SEQ ID NO: 37 - protein, 12 aa, artificial sequence
  synthetic peptide
ALARGDLGLSAG

SEQ ID NO: 38 - DNA, 36 bp, artificial sequence
  synthetic polynucleotide
gcgctggccaggggcgacctgggcctgagcgcgggc

SEQ ID NO: 39 - protein, 12 aa, artificial sequence
  synthetic peptide
AKARGDLGLSAK

SEQ ID NO: 40 - DNA, 357 bp, artificial sequence
  synthetic polynucleotide
gtggccacagaacagtacggcgtggtggccgataacctgcaacagcaaaacgcgaaggccaggggcgacctgggcctgagcgcgaaggccgctcctattgtaggggccgtcaatagtcaaggagccttacctggcatggtgtggcagaacagagatgtgtacctgcaaggacccatttgggccaaaattcctcacacggacggcaactttcacccttctccgctgatgggagggtttggaatgaagcacccgcctcctcagatcctcatcaaaaacacacctgtacctgcggatcctccaacggccttcaacaaggacaagctgaactctttcatcacccagtattctactggccaa

SEQ ID NO: 41 - DNA, 1068 bp, artificial sequence
  synthetic polynucleotide
ctcccgtacgtgctcgggtcggctcacgagggctgcctcccgccgttcccagcggacgttttcatgattcctcagtacgggtatctgacgcttaatgatggaagccaggccgtgggtcgttcgtccttttactgcctggaatatttcccgtcgcaaatgctaagaacgggtaacaacttccagttcagctacgagtttgagaacgtacctttccatagcagctacgctcacagccaaagcctggaccgactaatgaatccactcatcgaccaatacttgtactatctctcaaagactattaacggttctggacagaatcaacaaacgctaaaattcagtgtggccggacccagcaacatggctgtccagggaagaaactacatacctggacccagctaccgacaacaacgtgtctcaaccactgtgactcaaaacaacaacagcgaatttgcttggcctggagcttcttcttgggctctcaatggacgtaatagcttgatgaatcctggacctgctatggccagccacaaagaaggagaggaccgtttctttcctttgtctggatctttaatttttggcaaacaaggaactggaagagacaacgtggatgcggacaaagtcatgataaccaacgaagaagaaattaaaactactaacccggtagcaacggagtcctatggacaagtggccacaaaccaccagagtgcccaagcggccgccaggggcgacctgggcctgagctccggagcacaggcgcagaccggctgggttcaaaaccaaggaatacttccgggtatggtttggcaggacagagatgtgtacctgcaaggacccatttgggccaaaattcctcacacggacggcaactttcacccttctccgctgatgggagggtttggaatgaagcacccgcctcctcagatcctcatcaaaaacacacctgtacctgcggatcctccaacggccttcaacaaggacaagctgaactctttcatcacccagtattctactggccaagtcagcgtggagatcgagtgggagctgcagaaggaaaacagcaagcgctgg

SEQ ID NO: 42 - DNA, 1905 bp, artificial sequence
  synthetic polynucleotide
ccgtacgttctcggctctgcccaccagggctgcctgcctccgttcccggcggacgtgttcatgattccccagtacggctacctaacactcaacaacggtagtcaggccgtgggacgctcctccttctactgcctggaatactttccttcgcagatgctgagaaccggcaacaacttccagtttacttacaccttcgaggacgtgcctttccacagcagctacgcccacagccagagcttggaccggctgatgaatcctctgattgaccagtacctgtactacttgtctcggactcaaacaacaggaggcacggcaaatacgcagactctgggcttcagccaaggtgggcctaatacaatggccaatcaggcaaagaactggctgccaggaccctgttaccgccaacaacgcgtctcaacgacaaccgggcaaaacaacaatagcaactttgcctggactgctgggaccaaataccatctgaatggaagaaattcattggctaatcctggcatcgctatggcaacacacaaagacgacgaggagcgtttttttcccagtaacgggatcctgatttttggcaaacaaaatgctgccagagacaatgcggattacagcgatgtcatgctcaccagcgaggaagaaatcaaaaccactaaccctgtggctacagaggaatacggtatcgtggcagataacttgcagcagcaaaacgcggccgccaggggcgacctgggcctgagctccggaacggctcctcaaattggaactgtcaacagccagggggccttacccggtatggtctggcagaaccgggacgtgtacctgcagggtcccatctgccgtacgttctcggctctgcccaccagggctgcctgcctccgttcccggcggacgtgttcatgattccccagtacggctacctaacactcaacaacggtagtcaggccgtgggacgctcctccttctactgcctggaatactttccttcgcagatgctgagaaccggcaacaacttccagtttacttacaccttcgaggacgtgcctttccacagcagctacgcccacagccagagcttggaccggctgatgaatcctctgattgaccagtacctgtactacttgtctcggactcaaacaacaggaggcacggcaaatacgcagactctgggcttcagccaaggtgggcctaatacaatggccaatcaggcaaagaactggctgccaggaccctgttaccgccaacaacgcgtctcaacgacaaccgggcaaaacaacaatagcaactttgcctggactgctgggaccaaataccatctgaatggaagaaattcattggctaatcctggcatcgctatggcaacacacaaagacgacgaggagcgtttttttcccagtaacgggatcctgatttttggcaaacaaaatgctgccagagacaatgcggattacagcgatgtcatgctcaccagcgaggaagaaatcaaaaccactaaccctgtggctacagaggaatacggtatcgtggcagataacttgcagcagcaaaacgcggccgccaggggcgacctgggcctgagctccggaacggctcctcaaattggaactgtcaacagccagggggccttacccggtatggtctggcagaaccgggacgtgtacctgcagggtcccatcggccaagattcctcacacggacggcaacttccacccgtctccgctgatgggcggctttggcctgaaacatcctccgcctcagatcctgatcaagaacacgcctgtacctgcggatcctccgaccaccttcaaccagtcaaagctgaactctttcatcacgcaatacagcaccggacaggtcagcgtggaaattgaatgggagctgcagaaggaaaacagcaagcgctgg